European Patent Specification EP 3 426 680 B1, published August 14, 2024. Title: ACTIVIN TYPE 2 RECEPTOR BINDING PROTEINS AND USES THEREOF. Applicant: ACCELERON PHARMA KUMAR, RAVINDRA BELK, JONATHAN GRINBERG, ASYA SAKO, DIANNE CASTONGUY, ROSELYNE. The sequence listing filed with the application follows.

SEQUENCE LISTING (177 sequences)

SEQ ID NO: 1 - DNA, 390 bp, Homo sapian
cagctgcagctgcaggagtcgggcccaggactggtgaagccttcggagaccctgtccctcacctgcactgtctctggtggctccatcagcagtagtagttacgcatggggctggatccgccagcccccagggaaggggctggagtggattgggagtatctattatagtgggagcacctactacaacccgtccctcaagagtcgagtcaccatatccgtagacacgtccaagaaccagttctccctgaagctgagttctgtgaccgccgcagacacggcggtgtactactgcgccagagactcaggaataggatacagctacgcctcatcacatggctactactactacatggacgtatggggcaagggtacaactgtcaccgtctcctca

SEQ ID NO: 2 - protein, 130 aa, Homo sapian
QLQLQESGPGLVKPSETLSLTCTVSGGSISSSSYAWGWIRQPPGKGLEWIGSIYYSGSTYYNPSLKSRVTISVDTSKNQFSLKLSSVTAADTAVYYCARDSGIGYSYASSHGYYYYMDVWGKGTTVTVSS

SEQ ID NO: 3 - protein, 9 aa, Homo sapian
GGSISSSSY

SEQ ID NO: 4 - protein, 5 aa, Homo sapian
YYSGS

SEQ ID NO: 5 - protein, 20 aa, Homo sapian
DSGIGYSYASSHGYYYYMDV

SEQ ID NO: 6 - DNA, 1380 bp, Homo sapian
cagctgcagctgcaggagtcgggcccaggactggtgaagccttcggagaccctgtccctcacctgcactgtctctggtggctccatcagcagtagtagttacgcatggggctggatccgccagcccccagggaaggggctggagtggattgggagtatctattatagtgggagcacctactacaacccgtccctcaagagtcgagtcaccatatccgtagacacgtccaagaaccagttctccctgaagctgagttctgtgaccgccgcagacacggcggtgtactactgcgccagagactcaggaataggatacagctacgcctcatcacatggctactactactacatggacgtatggggcaagggtacaactgtcaccgtctcctcagctagcacaaaaggaccaagcgtgtttccactggcacctagcagcaaatccaccagcggcggaacagcagccctcgggtgcctggtgaaggattacttccctgagccagtcacagtgtcctggaactccggagccctgacatccggcgtgcacaccttccccgctgtgctgcaatccagcggactgtatagcctcagctccgtcgtgacagtcccttccagcagcctgggcacacagacttacatttgcaacgtgaaccacaaaccttccaacactaaggtggacaaaaaggtggaacccaaatcctgtgataagacccatacatgcccaccttgtcccgctcctgagctgctggggggaccttccgtctttctgtttcctccaaaaccaaaagacacactcatgatcagccggacccccgaagtcacctgtgtggtggtggacgtcagccacgaagatccagaggtcaagttcaattggtacgtggatggagtggaagtccacaacgcaaaaaccaaacctagagaagaacagtacaatagcacatacagggtggtgtccgtcctgacagtgctccaccaggactggctcaatggcaaagagtataagtgcaaggtgagcaacaaggccctgcctgcaccaattgagaaaacaattagcaaggcaaaggggcagccacgggaaccccaggtgtataccctgcccccaagccgggatgaactgaccaaaaaccaggtcagcctgacatgcctggtgaaagggttttacccaagcgatattgccgtcgagtgggagagcaacggacagccagaaaacaattacaaaaccaccccacctgtgctggactccgatgggagctttttcctgtacagcaagctcacagtggacaagtccagatggcaacagggcaacgtgttttcctgctccgtgatgcacgaggccctccacaaccactatacacaaaagtccctctccctcagcccaggaaag

SEQ ID NO: 7 - protein, 460 aa, Homo sapian
QLQLQESGPGLVKPSETLSLTCTVSGGSISSSSYAWGWIRQPPGKGLEWIGSIYYSGSTYYNPSLKSRVTISVDTSKNQFSLKLSSVTAADTAVYYCARDSGIGYSYASSHGYYYYMDVWGKGTTVTVSSASTKGPSVFPLAPSSKSTSGGTAALGCLVKDYFPEPVTVSWNSGALTSGVHTFPAVLQSSGLYSLSSVVTVPSSSLGTQTYICNVNHKPSNTKVDKKVEPKSCDKTHTCPPCPAPELLGGPSVFLFPPKPKDTLMISRTPEVTCVVVDVSHEDPEVKFNWYVDGVEVHNAKTKPREEQYNSTYRVVSVLTVLHQDWLNGKEYKCKVSNKALPAPIEKTISKAKGQPREPQVYTLPPSRDELTKNQVSLTCLVKGFYPSDIAVEWESNGQPENNYKTTPPVLDSDGSFFLYSKLTVDKSRWQQGNVFSCSVMHEALHNHYTQKSLSLSPGK

SEQ ID NO: 8 - DNA, 321 bp, Homo sapian
gaaatagtgttgacgcagtctccagccaccctgtctgtgtctccaggggaaagagccaccctctcctgcagggccagtcagagtgttggcagcaacttagcctggtaccagcagaaacctggccaggctcccaggctcctcatctatggtgcatccaccagggccactggtatcccagccaggttcagtggcagtgggtctgggacagagttcactctcaccatcagcagcctgcagtctgaagattttgcagtttattactgtcagcagtacttccacttccctctcacttttggcggagggaccaaggttgagatcaaa

SEQ ID NO: 9 - protein, 107 aa, Homo sapian
EIVLTQSPATLSVSPGERATLSCRASQSVGSNLAWYQQKPGQAPRLLIYGASTRATGIPARFSGSGSGTEFTLTISSLQSEDFAVYYCQQYFHFPLTFGGGTKVEIK

SEQ ID NO: 10 - protein, 11 aa, Homo sapian
RASQSVGSNLA

SEQ ID NO: 11 - protein, 7 aa, Homo sapian
GASTRAT

SEQ ID NO: 12 - protein, 9 aa, Homo sapian
QQYFHFPLT

SEQ ID NO: 13 - DNA, 642 bp, Homo sapian
gaaatagtgttgacgcagtctccagccaccctgtctgtgtctccaggggaaagagccaccctctcctgcagggccagtcagagtgttggcagcaacttagcctggtaccagcagaaacctggccaggctcccaggctcctcatctatggtgcatccaccagggccactggtatcccagccaggttcagtggcagtgggtctgggacagagttcactctcaccatcagcagcctgcagtctgaagattttgcagtttattactgtcagcagtacttccacttccctctcacttttggcggagggaccaaggttgagatcaaacgtacggtggctgcaccttccgtctttatctttccaccttccgatgagcagctgaagagcggaacagcaagcgtggtgtgtctgctgaacaacttttatccccgggaggcaaaggtgcagtggaaagtcgacaatgctctccagtccggcaattcccaagagagcgtgacagagcaagattccaaggactccacttacagcctgtccagcaccctcacactgagcaaggctgattacgagaaacacaaagtgtacgcttgtgaagtcacccaccaaggcctgagcagcccagtcactaagtcctttaaccggggcgaatgt

SEQ ID NO: 14 - protein, 214 aa, Homo sapian
EIVLTQSPATLSVSPGERATLSCRASQSVGSNLAWYQQKPGQAPRLLIYGASTRATGIPARFSGSGSGTEFTLTISSLQSEDFAVYYCQQYFHFPLTFGGGTKVEIKRTVAAPSVFIFPPSDEQLKSGTASVVCLLNNFYPREAKVQWKVDNALQSGNSQESVTEQDSKDSTYSLSSTLTLSKADYEKHKVYACEVTHQGLSSPVTKSFNRGEC

SEQ ID NO: 15 - DNA, 390 bp, Homo sapian
caggtgcagctgcaggagtcgggcccaggactggtgaagccttcacagaccctgtccctcacctgtactgtctctggtggctccatcgggagtggtggttactactggagctggatccgccagcacccagggaagggcctggagtggattggggggatctatggtagtgggagcacctactacaacccgtccctcaagagtcgagttaccatatcagtagacacgtctaagaaccagttctccctgaagctgagttctgtgaccgccgcagacacggcggtgtactactgcgccagagactcaggaataggatacagctacgcctcatcacatggctactactactacatggacgtatggggcaagggtacaactgtcaccgtctcctca

SEQ ID NO: 16 - protein, 130 aa, Homo sapian
QVQLQESGPGLVKPSQTLSLTCTVSGGSIGSGGYYWSWIRQHPGKGLEWIGGIYGSGSTYYNPSLKSRVTISVDTSKNQFSLKLSSVTAADTAVYYCARDSGIGYSYASSHGYYYYMDVWGKGTTVTVSS

SEQ ID NO: 17 - protein, 9 aa, Homo sapian
GGSIGSGGY

SEQ ID NO: 18 - protein, 4 aa, Homo sapian
YGSG

SEQ ID NO: 19 - DNA, 1380 bp, Homo sapian
caggtgcagctgcaggagtcgggcccaggactggtgaagccttcacagaccctgtccctcacctgtactgtctctggtggctccatcgggagtggtggttactactggagctggatccgccagcacccagggaagggcctggagtggattggggggatctatggtagtgggagcacctactacaacccgtccctcaagagtcgagttaccatatcagtagacacgtctaagaaccagttctccctgaagctgagttctgtgaccgccgcagacacggcggtgtactactgcgccagagactcaggaataggatacagctacgcctcatcacatggctactactactacatggacgtatggggcaagggtacaactgtcaccgtctcctcagctagcacaaaaggaccaagcgtgtttccactggcacctagcagcaaatccaccagcggcggaacagcagccctcgggtgcctggtgaaggattacttccctgagccagtcacagtgtcctggaactccggagccctgacatccggcgtgcacaccttccccgctgtgctgcaatccagcggactgtatagcctcagctccgtcgtgacagtcccttccagcagcctgggcacacagacttacatttgcaacgtgaaccacaaaccttccaacactaaggtggacaaaaaggtggaacccaaatcctgtgataagacccatacatgcccaccttgtcccgctcctgagctgctggggggaccttccgtctttctgtttcctccaaaaccaaaagacacactcatgatcagccggacccccgaagtcacctgtgtggtggtggacgtcagccacgaagatccagaggtcaagttcaattggtacgtggatggagtggaagtccacaacgcaaaaaccaaacctagagaagaacagtacaatagcacatacagggtggtgtccgtcctgacagtgctccaccaggactggctcaatggcaaagagtataagtgcaaggtgagcaacaaggccctgcctgcaccaattgagaaaacaattagcaaggcaaaggggcagccacgggaaccccaggtgtataccctgcccccaagccgggatgaactgaccaaaaaccaggtcagcctgacatgcctggtgaaagggttttacccaagcgatattgccgtcgagtgggagagcaacggacagccagaaaacaattacaaaaccaccccacctgtgctggactccgatgggagctttttcctgtacagcaagctcacagtggacaagtccagatggcaacagggcaacgtgttttcctgctccgtgatgcacgaggccctccacaaccactatacacaaaagtccctctccctcagcccaggaaag

SEQ ID NO: 20 - protein, 460 aa, Homo sapian
QVQLQESGPGLVKPSQTLSLTCTVSGGSIGSGGYYWSWIRQHPGKGLEWIGGIYGSGSTYYNPSLKSRVTISVDTSKNQFSLKLSSVTAADTAVYYCARDSGIGYSYASSHGYYYYMDVWGKGTTVTVSSASTKGPSVFPLAPSSKSTSGGTAALGCLVKDYFPEPVTVSWNSGALTSGVHTFPAVLQSSGLYSLSSVVTVPSSSLGTQTYICNVNHKPSNTKVDKKVEPKSCDKTHTCPPCPAPELLGGPSVFLFPPKPKDTLMISRTPEVTCVVVDVSHEDPEVKFNWYVDGVEVHNAKTKPREEQYNSTYRVVSVLTVLHQDWLNGKEYKCKVSNKALPAPIEKTISKAKGQPREPQVYTLPPSRDELTKNQVSLTCLVKGFYPSDIAVEWESNGQPENNYKTTPPVLDSDGSFFLYSKLTVDKSRWQQGNVFSCSVMHEALHNHYTQKSLSLSPGK

SEQ ID NO: 21 - DNA, 390 bp, Homo sapian
caggtgcagctgcaggagtcgggcccaggactggtgaagccttcacagaccctgtccctcacctgtactgtctctggtggctccatcaagagtggtgggtactactggagctggatccgccagcacccagggaagggcctggagtggattggggggatctatccgagtgggagcacctactacaacccgtccctcaagagtcgagttaccatatcagtagacacgtctaagaaccagttctccctgaagctgagttctgtgaccgccgcagacacggcggtgtactactgcgccagagactcaggaataggatacagctacgcctcatcacatggctactactactacatggacgtatggggcaagggtacaactgtcaccgtctcctca

SEQ ID NO: 22 - protein, 130 aa, Homo sapian
QVQLQESGPGLVKPSQTLSLTCTVSGGSIKSGGYYWSWIRQHPGKGLEWIGGIYPSGSTYYNPSLKSRVTISVDTSKNQFSLKLSSVTAADTAVYYCARDSGIGYSYASSHGYYYYMDVWGKGTTVTVSS

SEQ ID NO: 23 - protein, 9 aa, Homo sapian
GGSIKSGGY

SEQ ID NO: 24 - protein, 13 aa, Homo sapian
WIGGIYPSGSTYY

SEQ ID NO: 25 - DNA, 1380 bp, Homo sapian
caggtgcagctgcaggagtcgggcccaggactggtgaagccttcacagaccctgtccctcacctgtactgtctctggtggctccatcaagagtggtgggtactactggagctggatccgccagcacccagggaagggcctggagtggattggggggatctatccgagtgggagcacctactacaacccgtccctcaagagtcgagttaccatatcagtagacacgtctaagaaccagttctccctgaagctgagttctgtgaccgccgcagacacggcggtgtactactgcgccagagactcaggaataggatacagctacgcctcatcacatggctactactactacatggacgtatggggcaagggtacaactgtcaccgtctcctcagctagcacaaaaggaccaagcgtgtttccactggcacctagcagcaaatccaccagcggcggaacagcagccctcgggtgcctggtgaaggattacttccctgagccagtcacagtgtcctggaactccggagccctgacatccggcgtgcacaccttccccgctgtgctgcaatccagcggactgtatagcctcagctccgtcgtgacagtcccttccagcagcctgggcacacagacttacatttgcaacgtgaaccacaaaccttccaacactaaggtggacaaaaaggtggaacccaaatcctgtgataagacccatacatgcccaccttgtcccgctcctgagctgctggggggaccttccgtctttctgtttcctccaaaaccaaaagacacactcatgatcagccggacccccgaagtcacctgtgtggtggtggacgtcagccacgaagatccagaggtcaagttcaattggtacgtggatggagtggaagtccacaacgcaaaaaccaaacctagagaagaacagtacaatagcacatacagggtggtgtccgtcctgacagtgctccaccaggactggctcaatggcaaagagtataagtgcaaggtgagcaacaaggccctgcctgcaccaattgagaaaacaattagcaaggcaaaggggcagccacgggaaccccaggtgtataccctgcccccaagccgggatgaactgaccaaaaaccaggtcagcctgacatgcctggtgaaagggttttacccaagcgatattgccgtcgagtgggagagcaacggacagccagaaaacaattacaaaaccaccccacctgtgctggactccgatgggagctttttcctgtacagcaagctcacagtggacaagtccagatggcaacagggcaacgtgttttcctgctccgtgatgcacgaggccctccacaaccactatacacaaaagtccctctccctcagcccaggaaag

SEQ ID NO: 26 - protein, 460 aa, Homo sapian
QVQLQESGPGLVKPSQTLSLTCTVSGGSIKSGGYYWSWIRQHPGKGLEWIGGIYPSGSTYYNPSLKSRVTISVDTSKNQFSLKLSSVTAADTAVYYCARDSGIGYSYASSHGYYYYMDVWGKGTTVTVSSASTKGPSVFPLAPSSKSTSGGTAALGCLVKDYFPEPVTVSWNSGALTSGVHTFPAVLQSSGLYSLSSVVTVPSSSLGTQTYICNVNHKPSNTKVDKKVEPKSCDKTHTCPPCPAPELLGGPSVFLFPPKPKDTLMISRTPEVTCVVVDVSHEDPEVKFNWYVDGVEVHNAKTKPREEQYNSTYRVVSVLTVLHQDWLNGKEYKCKVSNKALPAPIEKTISKAKGQPREPQVYTLPPSRDELTKNQVSLTCLVKGFYPSDIAVEWESNGQPENNYKTTPPVLDSDGSFFLYSKLTVDKSRWQQGNVFSCSVMHEALHNHYTQKSLSLSPGK

SEQ ID NO: 27 - DNA, 390 bp, Homo sapian
caggtgcagctgcaggagtcgggcccaggactggtgaagccttcacagaccctgtccctcacctgtactgtctctggtggctccatcgagagcggtggttactactggagctggatccgccagcacccagggaagggcctggagtggattgggggtatctatgggagtgggagcacctactacaacccgtccctcaagagtcgagttaccatatcagtagacacgtctaagaaccagttctccctgaagctgagttctgtgaccgccgcagacacggcggtgtactactgcgccagagactcaggaataggatacagctacgcctcatcacatggctactactactacatggacgtatggggcaagggtacaactgtcaccgtctcctca

SEQ ID NO: 28 - protein, 130 aa, Homo sapian
QVQLQESGPGLVKPSQTLSLTCTVSGGSILSGGYYWSWIRQHPGKGLEWIGGIYYSGKTYYNPSLKSRVTISVDTSKNQFSLKLSSVTAADTAVYYCARDSGIGYSYASSHGYYYYMDVWGKGTTVTVSS

SEQ ID NO: 29 - protein, 9 aa, Homo sapian
GGSILSGGY

SEQ ID NO: 30 - protein, 5 aa, Homo sapian
YYSGK

SEQ ID NO: 31 - DNA, 1380 bp, Homo sapian
caggtgcagctgcaggagtcgggcccaggactggtgaagccttcacagaccctgtccctcacctgtactgtctctggtggctccatcgagagcggtggttactactggagctggatccgccagcacccagggaagggcctggagtggattgggggtatctatgggagtgggagcacctactacaacccgtccctcaagagtcgagttaccatatcagtagacacgtctaagaaccagttctccctgaagctgagttctgtgaccgccgcagacacggcggtgtactactgcgccagagactcaggaataggatacagctacgcctcatcacatggctactactactacatggacgtatggggcaagggtacaactgtcaccgtctcctcagctagcacaaaaggaccaagcgtgtttccactggcacctagcagcaaatccaccagcggcggaacagcagccctcgggtgcctggtgaaggattacttccctgagccagtcacagtgtcctggaactccggagccctgacatccggcgtgcacaccttccccgctgtgctgcaatccagcggactgtatagcctcagctccgtcgtgacagtcccttccagcagcctgggcacacagacttacatttgcaacgtgaaccacaaaccttccaacactaaggtggacaaaaaggtggaacccaaatcctgtgataagacccatacatgcccaccttgtcccgctcctgagctgctggggggaccttccgtctttctgtttcctccaaaaccaaaagacacactcatgatcagccggacccccgaagtcacctgtgtggtggtggacgtcagccacgaagatccagaggtcaagttcaattggtacgtggatggagtggaagtccacaacgcaaaaaccaaacctagagaagaacagtacaatagcacatacagggtggtgtccgtcctgacagtgctccaccaggactggctcaatggcaaagagtataagtgcaaggtgagcaacaaggccctgcctgcaccaattgagaaaacaattagcaaggcaaaggggcagccacgggaaccccaggtgtataccctgcccccaagccgggatgaactgaccaaaaaccaggtcagcctgacatgcctggtgaaagggttttacccaagcgatattgccgtcgagtgggagagcaacggacagccagaaaacaattacaaaaccaccccacctgtgctggactccgatgggagctttttcctgtacagcaagctcacagtggacaagtccagatggcaacagggcaacgtgttttcctgctccgtgatgcacgaggccctccacaaccactatacacaaaagtccctctccctcagcccaggaaag

SEQ ID NO: 32 - protein, 460 aa, Homo sapian
QVQLQESGPGLVKPSQTLSLTCTVSGGSIESGGYYWSWIRQHPGKGLEWIGGIYGSGSTYYNPSLKSRVTISVDTSKNQFSLKLSSVTAADTAVYYCARDSGIGYSYASSHGYYYYMDVWGKGTTVTVSSASTKGPSVFPLAPSSKSTSGGTAALGCLVKDYFPEPVTVSWNSGALTSGVHTFPAVLQSSGLYSLSSVVTVPSSSLGTQTYICNVNHKPSNTKVDKKVEPKSCDKTHTCPPCPAPELLGGPSVFLFPPKPKDTLMISRTPEVTCVVVDVSHEDPEVKFNWYVDGVEVHNAKTKPREEQYNSTYRVVSVLTVLHQDWLNGKEYKCKVSNKALPAPIEKTISKAKGQPREPQVYTLPPSRDELTKNQVSLTCLVKGFYPSDIAVEWESNGQPENNYKTTPPVLDSDGSFFLYSKLTVDKSRWQQGNVFSCSVMHEALHNHYTQKSLSLSPGK

SEQ ID NO: 33 - DNA, 390 bp, Homo sapian
caggtgcagctgcaggagtcgggcccaggactggtgaagccttcacagaccctgtccctcacctgtactgtctctggtggctccatctctagtggtggttacttttggagctggatccgccagcacccagggaagggcctggagtggattggggggatctattacagtgggcggacctactacaacccgtccctcaagagtcgagttaccatatcagtagacacgtctaagaaccagttctccctgaagctgagttctgtgaccgccgcagacacggcggtgtactactgcgccagagactcaggaataggatacagctacgcctcatcacatggctactactactacatggacgtatggggcaagggtacaactgtcaccgtctcctca

SEQ ID NO: 34 - protein, 130 aa, Homo sapian
QVQLQESGPGLVKPSQTLSLTCTVSGGSISSGGYFWSWIRQHPGKGLEWIGGIYYSGRTYYNPSLKSRVTISVDTSKNQFSLKLSSVTAADTAVYYCARDSGIGYSYASSHGYYYYMDVWGKGTTVTVSS

SEQ ID NO: 35 - protein, 9 aa, Homo sapian
GGSISSGGY

SEQ ID NO: 36 - protein, 6 aa, Homo sapian
YYSGRT

SEQ ID NO: 37 - DNA, 1380 bp, Homo sapian
caggtgcagctgcaggagtcgggcccaggactggtgaagccttcacagaccctgtccctcacctgtactgtctctggtggctccatctctagtggtggttacttttggagctggatccgccagcacccagggaagggcctggagtggattggggggatctattacagtgggcggacctactacaacccgtccctcaagagtcgagttaccatatcagtagacacgtctaagaaccagttctccctgaagctgagttctgtgaccgccgcagacacggcggtgtactactgcgccagagactcaggaataggatacagctacgcctcatcacatggctactactactacatggacgtatggggcaagggtacaactgtcaccgtctcctcagctagcacaaaaggaccaagcgtgtttccactggcacctagcagcaaatccaccagcggcggaacagcagccctcgggtgcctggtgaaggattacttccctgagccagtcacagtgtcctggaactccggagccctgacatccggcgtgcacaccttccccgctgtgctgcaatccagcggactgtatagcctcagctccgtcgtgacagtcccttccagcagcctgggcacacagacttacatttgcaacgtgaaccacaaaccttccaacactaaggtggacaaaaaggtggaacccaaatcctgtgataagacccatacatgcccaccttgtcccgctcctgagctgctggggggaccttccgtctttctgtttcctccaaaaccaaaagacacactcatgatcagccggacccccgaagtcacctgtgtggtggtggacgtcagccacgaagatccagaggtcaagttcaattggtacgtggatggagtggaagtccacaacgcaaaaaccaaacctagagaagaacagtacaatagcacatacagggtggtgtccgtcctgacagtgctccaccaggactggctcaatggcaaagagtataagtgcaaggtgagcaacaaggccctgcctgcaccaattgagaaaacaattagcaaggcaaaggggcagccacgggaaccccaggtgtataccctgcccccaagccgggatgaactgaccaaaaaccaggtcagcctgacatgcctggtgaaagggttttacccaagcgatattgccgtcgagtgggagagcaacggacagccagaaaacaattacaaaaccaccccacctgtgctggactccgatgggagctttttcctgtacagcaagctcacagtggacaagtccagatggcaacagggcaacgtgttttcctgctccgtgatgcacgaggccctccacaaccactatacacaaaagtccctctccctcagcccaggaaag

SEQ ID NO: 38 - protein, 460 aa, Homo sapian
QVQLQESGPGLVKPSQTLSLTCTVSGGSISSGGYFWSWIRQHPGKGLEWIGGIYYSGRTYYNPSLKSRVTISVDTSKNQFSLKLSSVTAADTAVYYCARDSGIGYSYASSHGYYYYMDVWGKGTTVTVSSASTKGPSVFPLAPSSKSTSGGTAALGCLVKDYFPEPVTVSWNSGALTSGVHTFPAVLQSSGLYSLSSVVTVPSSSLGTQTYICNVNHKPSNTKVDKKVEPKSCDKTHTCPPCPAPELLGGPSVFLFPPKPKDTLMISRTPEVTCVVVDVSHEDPEVKFNWYVDGVEVHNAKTKPREEQYNSTYRVVSVLTVLHQDWLNGKEYKCKVSNKALPAPIEKTISKAKGQPREPQVYTLPPSRDELTKNQVSLTCLVKGFYPSDIAVEWESNGQPENNYKTTPPVLDSDGSFFLYSKLTVDKSRWQQGNVFSCSVMHEALHNHYTQKSLSLSPGK

SEQ ID NO: 39 - DNA, 390 bp, Homo sapian; identical to SEQ ID NO: 27

SEQ ID NO: 40 - protein, 130 aa, Homo sapian
QVQLQESGPGLVKPSQTLSLTCTVSGGSIESGGYYWSWIRQHPGKGLEWIGGIYGSGSTYYNPSLKSRVTISVDTSKNQFSLKLSSVTAADTAVYYCARDSGIGYSYASSHGYYYYMDVWGKGTTVTVSS

SEQ ID NO: 41 - protein, 9 aa, Homo sapian
GGSIESGGY

SEQ ID NO: 42 - DNA, 1380 bp, Homo sapian; identical to SEQ ID NO: 31

SEQ ID NO: 43 - protein, 460 aa, Homo sapian; identical to SEQ ID NO: 32

SEQ ID NO: 44 - DNA, 363 bp, Homo sapian
cagctgcagctgcaggagtcgggcccaggactggtgaagccttcggagaccctgtccctcacctgcactgtctctggtggctccatcagcagtagtagttacgcatggggctggatccgccagcccccagggaaggggctggagtggattgggagtatctattatagtgggagcacctactacaacccgtccctcaagagtcgagtcaccatatccgtagacacgtccaagaaccagttctccctgaagctgagttctgtgaccgccgcagacacggcggtgtactactgcgccagagctggaaaataccgatggcacggaatggacgtatggggccagggaacaactgtcaccgtctcctca

SEQ ID NO: 45 - protein, 121 aa, Homo sapian
QLQLQESGPGLVKPSETLSLTCTVSGGSISSSSYAWGWIRQPPGKGLEWIGSIYYSGSTYYNPSLKSRVTISVDTSKNQFSLKLSSVTAADTAVYYCARAGKYRWHGMDVWGQGTTVTVSS

SEQ ID NO: 46 - protein, 11 aa, Homo sapian
AGKYRWHGMDV

SEQ ID NO: 47 - DNA, 1353 bp, Homo sapian
cagctgcagctgcaggagtcgggcccaggactggtgaagccttcggagaccctgtccctcacctgcactgtctctggtggctccatcagcagtagtagttacgcatggggctggatccgccagcccccagggaaggggctggagtggattgggagtatctattatagtgggagcacctactacaacccgtccctcaagagtcgagtcaccatatccgtagacacgtccaagaaccagttctccctgaagctgagttctgtgaccgccgcagacacggcggtgtactactgcgccagagctggaaaataccgatggcacggaatggacgtatggggccagggaacaactgtcaccgtctcctcagctagcacaaaaggaccaagcgtgtttccactggcacctagcagcaaatccaccagcggcggaacagcagccctcgggtgcctggtgaaggattacttccctgagccagtcacagtgtcctggaactccggagccctgacatccggcgtgcacaccttccccgctgtgctgcaatccagcggactgtatagcctcagctccgtcgtgacagtcccttccagcagcctgggcacacagacttacatttgcaacgtgaaccacaaaccttccaacactaaggtggacaaaaaggtggaacccaaatcctgtgataagacccatacatgcccaccttgtcccgctcctgagctgctggggggaccttccgtctttctgtttcctccaaaaccaaaagacacactcatgatcagccggacccccgaagtcacctgtgtggtggtggacgtcagccacgaagatccagaggtcaagttcaattggtacgtggatggagtggaagtccacaacgcaaaaaccaaacctagagaagaacagtacaatagcacatacagggtggtgtccgtcctgacagtgctccaccaggactggctcaatggcaaagagtataagtgcaaggtgagcaacaaggccctgcctgcaccaattgagaaaacaattagcaaggcaaaggggcagccacgggaaccccaggtgtataccctgcccccaagccgggatgaactgaccaaaaaccaggtcagcctgacatgcctggtgaaagggttttacccaagcgatattgccgtcgagtgggagagcaacggacagccagaaaacaattacaaaaccaccccacctgtgctggactccgatgggagctttttcctgtacagcaagctcacagtggacaagtccagatggcaacagggcaacgtgttttcctgctccgtgatgcacgaggccctccacaaccactatacacaaaagtccctctccctcagcccaggaaag

SEQ ID NO: 48 - protein, 451 aa, Homo sapian
QLQLQESGPGLVKPSETLSLTCTVSGGSISSSSYAWGWIRQPPGKGLEWIGSIYYSGSTYYNPSLKSRVTISVDTSKNQFSLKLSSVTAADTAVYYCARAGKYRWHGMDVWGQGTTVTVSSASTKGPSVFPLAPSSKSTSGGTAALGCLVKDYFPEPVTVSWNSGALTSGVHTFPAVLQSSGLYSLSSVVTVPSSSLGTQTYICNVNHKPSNTKVDKKVEPKSCDKTHTCPPCPAPELLGGPSVFLFPPKPKDTLMISRTPEVTCVVVDVSHEDPEVKFNWYVDGVEVHNAKTKPREEQYNSTYRVVSVLTVLHQDWLNGKEYKCKVSNKALPAPIEKTISKAKGQPREPQVYTLPPSRDELTKNQVSLTCLVKGFYPSDIAVEWESNGQPENNYKTTPPVLDSDGSFFLYSKLTVDKSRWQQGNVFSCSVMHEALHNHYTQKSLSLSPGK

SEQ ID NO: 49 - DNA, 321 bp, Homo sapian
gacatccagatgacccagtctccatcttccgtgtctgcatctgtaggagacagagtcaccatcacttgtcgggcgagtcagggtattagcagctggttagcctggtatcagcagaaaccagggaaagcccctaagctcctgatctatgctgcatccaatttgcaaagtggggtcccatcaaggttcagcggcagtggatctgggacagatttcactctcaccatcagcagcctgcagcctgaagattttgcaacttattactgtcagcaggcacccgacctccctatcacttttggcggagggaccaaggttgagatcaaa

SEQ ID NO: 50 - protein, 107 aa, Homo sapian
DIQMTQSPSSVSASVGDRVTITCRASQGISSWLAWYQQKPGKAPKLLIYAASNLQSGVPSRFSGSGSGTDFTLTISSLQPEDFATYYCQQAPDLPITFGGGTKVEIK

SEQ ID NO: 51 - protein, 11 aa, Homo sapian
RASQGISSWLA

SEQ ID NO: 52 - protein, 7 aa, Homo sapian
AASNLQS

SEQ ID NO: 53 - protein, 9 aa, Homo sapian
QQAPDLPIT

SEQ ID NO: 54 - DNA, 642 bp, Homo sapian
gacatccagatgacccagtctccatcttccgtgtctgcatctgtaggagacagagtcaccatcacttgtcgggcgagtcagggtattagcagctggttagcctggtatcagcagaaaccagggaaagcccctaagctcctgatctatgctgcatccaatttgcaaagtggggtcccatcaaggttcagcggcagtggatctgggacagatttcactctcaccatcagcagcctgcagcctgaagattttgcaacttattactgtcagcaggcacccgacctccctatcacttttggcggagggaccaaggttgagatcaaacgtacggtggctgcaccttccgtctttatctttccaccttccgatgagcagctgaagagcggaacagcaagcgtggtgtgtctgctgaacaacttttatccccgggaggcaaaggtgcagtggaaagtcgacaatgctctccagtccggcaattcccaagagagcgtgacagagcaagattccaaggactccacttacagcctgtccagcaccctcacactgagcaaggctgattacgagaaacacaaagtgtacgcttgtgaagtcacccaccaaggcctgagcagcccagtcactaagtcctttaaccggggcgaatgt

SEQ ID NO: 55 - protein, 214 aa, Homo sapian
DIQMTQSPSSVSASVGDRVTITCRASQGISSWLAWYQQKPGKAPKLLIYAASNLQSGVPSRFSGSGSGTDFTLTISSLQPEDFATYYCQQAPDLPITFGGGTKVEIKRTVAAPSVFIFPPSDEQLKSGTASVVCLLNNFYPREAKVQWKVDNALQSGNSQESVTEQDSKDSTYSLSSTLTLSKADYEKHKVYACEVTHQGLSSPVTKSFNRGEC

SEQ ID NO: 56 - DNA, 360 bp, Homo sapian
caggtgcagctgcaggagtcgggcccaggactggtgaagccttcggagaccctgtccctcacctgcgctgtctctggttactccatcagcagtggtgtttactggatgtggatccggcagcccccagggaaggggctggagtggattgggagtatcgttcatagtgggcatacctactacaacccgtccctcaagagtcgagtcaccatatcagtagacacgtccaagaaccagttctccctgaagctgagttctgtgaccgccgcagacacggcggtgtactactgcgccagagctggaaaataccgatggcacggaatggacgtatggggccagggaacaactgtcaccgtctcctca

SEQ ID NO: 57 - protein, 120 aa, Homo sapian
QVQLQESGPGLVKPSETLSLTCAVSGYSISSGVYWMWIRQPPGKGLEWIGSIVHSGHTYYNPSLKSRVTISVDTSKNQFSLKLSSVTAADTAVYYCARAGKYRWHGMDVWGQGTTVTVSS

SEQ ID NO: 58 - protein, 8 aa, Homo sapian
GYSISSGV

SEQ ID NO: 59 - protein, 5 aa, Homo sapian
VHSGH

SEQ ID NO: 60 - DNA, 1350 bp, Homo sapian
caggtgcagctgcaggagtcgggcccaggactggtgaagccttcggagaccctgtccctcacctgcgctgtctctggttactccatcagcagtggtgtttactggatgtggatccggcagcccccagggaaggggctggagtggattgggagtatcgttcatagtgggcatacctactacaacccgtccctcaagagtcgagtcaccatatcagtagacacgtccaagaaccagttctccctgaagctgagttctgtgaccgccgcagacacggcggtgtactactgcgccagagctggaaaataccgatggcacggaatggacgtatggggccagggaacaactgtcaccgtctcctcagctagcacaaaaggaccaagcgtgtttccactggcacctagcagcaaatccaccagcggcggaacagcagccctcgggtgcctggtgaaggattacttccctgagccagtcacagtgtcctggaactccggagccctgacatccggcgtgcacaccttccccgctgtgctgcaatccagcggactgtatagcctcagctccgtcgtgacagtcccttccagcagcctgggcacacagacttacatttgcaacgtgaaccacaaaccttccaacactaaggtggacaaaaaggtggaacccaaatcctgtgataagacccatacatgcccaccttgtcccgctcctgagctgctggggggaccttccgtctttctgtttcctccaaaaccaaaagacacactcatgatcagccggacccccgaagtcacctgtgtggtggtggacgtcagccacgaagatccagaggtcaagttcaattggtacgtggatggagtggaagtccacaacgcaaaaaccaaacctagagaagaacagtacaatagcacatacagggtggtgtccgtcctgacagtgctccaccaggactggctcaatggcaaagagtataagtgcaaggtgagcaacaaggccctgcctgcaccaattgagaaaacaattagcaaggcaaaggggcagccacgggaaccccaggtgtataccctgcccccaagccgggatgaactgaccaaaaaccaggtcagcctgacatgcctggtgaaagggttttacccaagcgatattgccgtcgagtgggagagcaacggacagccagaaaacaattacaaaaccaccccacctgtgctggactccgatgggagctttttcctgtacagcaagctcacagtggacaagtccagatggcaacagggcaacgtgttttcctgctccgtgatgcacgaggccctccacaaccactatacacaaaagtccctctccctcagcccaggaaag

SEQ ID NO: 61 - protein, 450 aa, Homo sapian
QVQLQESGPGLVKPSETLSLTCAVSGYSISSGVYWMWIRQPPGKGLEWIGSIVHSGHTYYNPSLKSRVTISVDTSKNQFSLKLSSVTAADTAVYYCARAGKYRWHGMDVWGQGTTVTVSSASTKGPSVFPLAPSSKSTSGGTAALGCLVKDYFPEPVTVSWNSGALTSGVHTFPAVLQSSGLYSLSSVVTVPSSSLGTQTYICNVNHKPSNTKVDKKVEPKSCDKTHTCPPCPAPELLGGPSVFLFPPKPKDTLMISRTPEVTCVVVDVSHEDPEVKFNWYVDGVEVHNAKTKPREEQYNSTYRVVSVLTVLHQDWLNGKEYKCKVSNKALPAPIEKTISKAKGQPREPQVYTLPPSRDELTKNQVSLTCLVKGFYPSDIAVEWESNGQPENNYKTTPPVLDSDGSFFLYSKLTVDKSRWQQGNVFSCSVMHEALHNHYTQKSLSLSPGK

SEQ ID NO: 62 - DNA, 363 bp, Homo sapian
gaggtgcagctgttggagtctgggggaggcttggtacagcctggggggtccctgagactctcctgtgcagcctctggattcacctttagcagctatgccatgagctgggtccgccaggctccagggaaggggctggagtgggtctcaggaattagtggtagtggtggtagcacatactacgcagactccgtgaagggccggttcaccatctccagagacaattccaagaacacgctgtatctgcaaatgaacagcctgagagccgaggacacggcggtgtactactgcgccaaggaccctttgtctctacttctaggctactttgactactggggacagggtgcattggtcaccgtctcctca

SEQ ID NO: 63 - protein, 121 aa, Homo sapian
EVQLLESGGGLVQPGGSLRLSCAASGFTFSSYAMSWVRQAPGKGLEWVSGISGSGGSTYYADSVKGRFTISRDNSKNTLYLQMNSLRAEDTAVYYCAKDPLSLLLGYFDYWGQGALVTVSS

SEQ ID NO: 64 - protein, 7 aa, Homo sapian
GFTFSSY

SEQ ID NO: 65 - protein, 6 aa, Homo sapian
SGSGGS

SEQ ID NO: 66 - protein, 12 aa, Homo sapian
DPLSLLLGYFDY

SEQ ID NO: 67 - DNA, 1353 bp, Homo sapian
gaggtgcagctgttggagtctgggggaggcttggtacagcctggggggtccctgagactctcctgtgcagcctctggattcacctttagcagctatgccatgagctgggtccgccaggctccagggaaggggctggagtgggtctcaggaattagtggtagtggtggtagcacatactacgcagactccgtgaagggccggttcaccatctccagagacaattccaagaacacgctgtatctgcaaatgaacagcctgagagccgaggacacggcggtgtactactgcgccaaggaccctttgtctctacttctaggctactttgactactggggacagggtgcattggtcaccgtctcctcagctagcacaaaaggaccaagcgtgtttccactggcacctagcagcaaatccaccagcggcggaacagcagccctcgggtgcctggtgaaggattacttccctgagccagtcacagtgtcctggaactccggagccctgacatccggcgtgcacaccttccccgctgtgctgcaatccagcggactgtatagcctcagctccgtcgtgacagtcccttccagcagcctgggcacacagacttacatttgcaacgtgaaccacaaaccttccaacactaaggtggacaaaaaggtggaacccaaatcctgtgataagacccatacatgcccaccttgtcccgctcctgagctgctggggggaccttccgtctttctgtttcctccaaaaccaaaagacacactcatgatcagccggacccccgaagtcacctgtgtggtggtggacgtcagccacgaagatccagaggtcaagttcaattggtacgtggatggagtggaagtccacaacgcaaaaaccaaacctagagaagaacagtacaatagcacatacagggtggtgtccgtcctgacagtgctccaccaggactggctcaatggcaaagagtataagtgcaaggtgagcaacaaggccctgcctgcaccaattgagaaaacaattagcaaggcaaaggggcagccacgggaaccccaggtgtataccctgcccccaagccgggatgaactgaccaaaaaccaggtcagcctgacatgcctggtgaaagggttttacccaagcgatattgccgtcgagtgggagagcaacggacagccagaaaacaattacaaaaccaccccacctgtgctggactccgatgggagctttttcctgtacagcaagctcacagtggacaagtccagatggcaacagggcaacgtgttttcctgctccgtgatgcacgaggccctccacaaccactatacacaaaagtccctctccctcagcccaggaaag

SEQ ID NO: 68 - protein, 451 aa, Homo sapian
EVQLLESGGGLVQPGGSLRLSCAASGFTFSSYAMSWVRQAPGKGLEWVSGISGSGGSTYYADSVKGRFTISRDNSKNTLYLQMNSLRAEDTAVYYCAKDPLSLLLGYFDYWGQGALVTVSSASTKGPSVFPLAPSSKSTSGGTAALGCLVKDYFPEPVTVSWNSGALTSGVHTFPAVLQSSGLYSLSSVVTVPSSSLGTQTYICNVNHKPSNTKVDKKVEPKSCDKTHTCPPCPAPELLGGPSVFLFPPKPKDTLMISRTPEVTCVVVDVSHEDPEVKFNWYVDGVEVHNAKTKPREEQYNSTYRVVSVLTVLHQDWLNGKEYKCKVSNKALPAPIEKTISKAKGQPREPQVYTLPPSRDELTKNQVSLTCLVKGFYPSDIAVEWESNGQPENNYKTTPPVLDSDGSFFLYSKLTVDKSRWQQGNVFSCSVMHEALHNHYTQKSLSLSPGK

SEQ ID NO: 69 - DNA, 321 bp, Homo sapian
gacatccagatgacccagtctccttccaccctgtctgcatctgtaggagacagagtcaccatcacttgccgggccagtcagagtattagtagctggttggcctggtatcagcagaaaccagggaaagcccctaagctcctgatctatgatgcctccagtttggaaagtggggtcccatcaaggttcagcggcagtggatctgggacagaattcactctcaccatcagcagcctgcagcctgatgattttgcaacttattactgccagcagtacaatcgccactctcctacttttggcggagggaccaaggttgagatcaaa

SEQ ID NO: 70 - protein, 107 aa, Homo sapian
DIQMTQSPSTLSASVGDRVTITCRASQSISSWLAWYQQKPGKAPKLLIYDASSLESGVPSRFSGSGSGTEFTLTISSLQPDDFATYYCQQYNRHSPTFGGGTKVEIK

SEQ ID NO: 71 - protein, 11 aa, Homo sapian
RASQSISSWLA

SEQ ID NO: 72 - protein, 7 aa, Homo sapian
DASSLES

SEQ ID NO: 73 - protein, 9 aa, Homo sapian
QQYNRHSPT

SEQ ID NO: 74 - DNA, 642 bp, Homo sapian
gacatccagatgacccagtctccttccaccctgtctgcatctgtaggagacagagtcaccatcacttgccgggccagtcagagtattagtagctggttggcctggtatcagcagaaaccagggaaagcccctaagctcctgatctatgatgcctccagtttggaaagtggggtcccatcaaggttcagcggcagtggatctgggacagaattcactctcaccatcagcagcctgcagcctgatgattttgcaacttattactgccagcagtacaatcgccactctcctacttttggcggagggaccaaggttgagatcaaacgtacggtggctgcaccttccgtctttatctttccaccttccgatgagcagctgaagagcggaacagcaagcgtggtgtgtctgctgaacaacttttatccccgggaggcaaaggtgcagtggaaagtcgacaatgctctccagtccggcaattcccaagagagcgtgacagagcaagattccaaggactccacttacagcctgtccagcaccctcacactgagcaaggctgattacgagaaacacaaagtgtacgcttgtgaagtcacccaccaaggcctgagcagcccagtcactaagtcctttaaccggggcgaatgt

SEQ ID NO: 75 - protein, 214 aa, Homo sapian
DIQMTQSPSTLSASVGDRVTITCRASQSISSWLAWYQQKPGKAPKLLIYDASSLESGVPSRFSGSGSGTEFTLTISSLQPDDFATYYCQQYNRHSPTFGGGTKVEIKRTVAAPSVFIFPPSDEQLKSGTASVVCLLNNFYPREAKVQWKVDNALQSGNSQESVTEQDSKDSTYSLSSTLTLSKADYEKHKVYACEVTHQGLSSPVTKSFNRGEC

SEQ ID NO: 76 - DNA, 363 bp, Homo sapian
gaggtgcagctgttggagtctgggggaggcttggtacagcctggggggtccctgagactctcctgtgcagcctctggattcacctttagccgttatgccatgtcgtgggtccgccaggctccagggaaggggctggagtgggtctcaggtattagtggaagtggtggtgcgacatactacgcagactccgtgaagggccggttcaccatctccagagacaattccaagaacacgctgtatctgcaaatgaacagcctgagagccgaggacacggcggtgtactactgcgccaaggaccctttgtctctacttctaggctactttgactactggggacagggtgcattggtcaccgtctcctca

SEQ ID NO: 77 - protein, 121 aa, Homo sapian
EVQLLESGGGLVQPGGSLRLSCAASGFTFSRYAMSWVRQAPGKGLEWVSGISGSGGATYYADSVKGRFTISRDNSKNTLYLQMNSLRAEDTAVYYCAKDPLSLLLGYFDYWGQGALVTVSS

SEQ ID NO: 78 - protein, 7 aa, Homo sapian
GFTFSRY

SEQ ID NO: 79 - protein, 6 aa, Homo sapian
SGSGGA

SEQ ID NO: 80 - protein, 12 aa, Homo sapian
DPLSLLLGYFDY

SEQ ID NO: 81 - DNA, 1353 bp, Homo sapian
gaggtgcagctgttggagtctgggggaggcttggtacagcctggggggtccctgagactctcctgtgcagcctctggattcacctttagccgttatgccatgtcgtgggtccgccaggctccagggaaggggctggagtgggtctcaggtattagtggaagtggtggtgcgacatactacgcagactccgtgaagggccggttcaccatctccagagacaattccaagaacacgctgtatctgcaaatgaacagcctgagagccgaggacacggcggtgtactactgcgccaaggaccctttgtctctacttctaggctactttgactactggggacagggtgcattggtcaccgtctcctcagctagcacaaaaggaccaagcgtgtttccactggcacctagcagcaaatccaccagcggcggaacagcagccctcgggtgcctggtgaaggattacttccctgagccagtcacagtgtcctggaactccggagccctgacatccggcgtgcacaccttccccgctgtgctgcaatccagcggactgtatagcctcagctccgtcgtgacagtcccttccagcagcctgggcacacagacttacatttgcaacgtgaaccacaaaccttccaacactaaggtggacaaaaaggtggaacccaaatcctgtgataagacccatacatgcccaccttgtcccgctcctgagctgctggggggaccttccgtctttctgtttcctccaaaaccaaaagacacactcatgatcagccggacccccgaagtcacctgtgtggtggtggacgtcagccacgaagatccagaggtcaagttcaattggtacgtggatggagtggaagtccacaacgcaaaaaccaaacctagagaagaacagtacaatagcacatacagggtggtgtccgtcctgacagtgctccaccaggactggctcaatggcaaagagtataagtgcaaggtgagcaacaaggccctgcctgcaccaattgagaaaacaattagcaaggcaaaggggcagccacgggaaccccaggtgtataccctgcccccaagccgggatgaactgaccaaaaaccaggtcagcctgacatgcctggtgaaagggttttacccaagcgatattgccgtcgagtgggagagcaacggacagccagaaaacaattacaaaaccaccccacctgtgctggactccgatgggagctttttcctgtacagcaagctcacagtggacaagtccagatggcaacagggcaacgtgttttcctgctccgtgatgcacgaggccctccacaaccactatacacaaaagtccctctccctcagcccaggaaag

SEQ ID NO: 82 - protein, 451 aa, Homo sapian
EVQLLESGGGLVQPGGSLRLSCAASGFTFSRYAMSWVRQAPGKGLEWVSGISGSGGATYYADSVKGRFTISRDNSKNTLYLQMNSLRAEDTAVYYCAKDPLSLLLGYFDYWGQGALVTVSSASTKGPSVFPLAPSSKSTSGGTAALGCLVKDYFPEPVTVSWNSGALTSGVHTFPAVLQSSGLYSLSSVVTVPSSSLGTQTYICNVNHKPSNTKVDKKVEPKSCDKTHTCPPCPAPELLGGPSVFLFPPKPKDTLMISRTPEVTCVVVDVSHEDPEVKFNWYVDGVEVHNAKTKPREEQYNSTYRVVSVLTVLHQDWLNGKEYKCKVSNKALPAPIEKTISKAKGQPREPQVYTLPPSRDELTKNQVSLTCLVKGFYPSDIAVEWESNGQPENNYKTTPPVLDSDGSFFLYSKLTVDKSRWQQGNVFSCSVMHEALHNHYTQKSLSLSPGK

SEQ ID NO: 83 - DNA, 360 bp, Homo sapian
caggttcagctggtgcagtctggagctgaggtgaagaagcctggggcctcagtgaaggtctcctgcaaggcttctggttacacctttaccagctatggtatcagctgggtgcgacaggcccctggacaagggcttgagtggatgggatggatcagcccttacaatggtaacacaaactatgcacagaagctccagggcagagtcaccatgaccacagacacatccacgagcacagcctacatggagctgaggagcctgagatctgacgacacggcggtgtactactgcgctagagtatctatgtacgccccagagccaatggacgtatggggccagggaacaactgtcaccgtctcctca

SEQ ID NO: 84 - protein, 120 aa, Homo sapian
QVQLVQSGAEVKKPGASVKVSCKASGYTFTSYGISWVRQAPGQGLEWMGWISPYNGNTNYAQKLQGRVTMTTDTSTSTAYMELRSLRSDDTAVYYCARVSMYAPEPMDVWGQGTTVTVSS

SEQ ID NO: 85 - protein, 7 aa, Homo sapian
GYTFTSY

SEQ ID NO: 86 - protein, 6 aa, Homo sapian
SPYNGN

SEQ ID NO: 87 - protein, 11 aa, Homo sapian
VSMYAPEPMDV

SEQ ID NO: 88 - DNA, 1350 bp, Homo sapian
caggttcagctggtgcagtctggagctgaggtgaagaagcctggggcctcagtgaaggtctcctgcaaggcttctggttacacctttaccagctatggtatcagctgggtgcgacaggcccctggacaagggcttgagtggatgggatggatcagcccttacaatggtaacacaaactatgcacagaagctccagggcagagtcaccatgaccacagacacatccacgagcacagcctacatggagctgaggagcctgagatctgacgacacggcggtgtactactgcgctagagtatctatgtacgccccagagccaatggacgtatggggccagggaacaactgtcaccgtctcctcagctagcacaaaaggaccaagcgtgtttccactggcacctagcagcaaatccaccagcggcggaacagcagccctcgggtgcctggtgaaggattacttccctgagccagtcacagtgtcctggaactccggagccctgacatccggcgtgcacaccttccccgctgtgctgcaatccagcggactgtatagcctcagctccgtcgtgacagtcccttccagcagcctgggcacacagacttacatttgcaacgtgaaccacaaaccttccaacactaaggtggacaaaaaggtggaacccaaatcctgtgataagacccatacatgcccaccttgtcccgctcctgagctgctggggggaccttccgtctttctgtttcctccaaaaccaaaagacacactcatgatcagccggacccccgaagtcacctgtgtggtggtggacgtcagccacgaagatccagaggtcaagttcaattggtacgtggatggagtggaagtccacaacgcaaaaaccaaacctagagaagaacagtacaatagcacatacagggtggtgtccgtcctgacagtgctccaccaggactggctcaatggcaaagagtataagtgcaaggtgagcaacaaggccctgcctgcaccaattgagaaaacaattagcaaggcaaaggggcagccacgggaaccccaggtgtataccctgcccccaagccgggatgaactgaccaaaaaccaggtcagcctgacatgcctggtgaaagggttttacccaagcgatattgccgtcgagtgggagagcaacggacagccagaaaacaattacaaaaccaccccacctgtgctggactccgatgggagctttttcctgtacagcaagctcacagtggacaagtccagatggcaacagggcaacgtgttttcctgctccgtgatgcacgaggccctccacaaccactatacacaaaagtccctctccctcagcccaggaaag

SEQ ID NO: 89 - protein, 450 aa, Homo sapian
QVQLVQSGAEVKKPGASVKVSCKASGYTFTSYGISWVRQAPGQGLEWMGWISPYNGNTNYAQKLQGRVTMTTDTSTSTAYMELRSLRSDDTAVYYCARVSMYAPEPMDVWGQGTTVTVSSASTKGPSVFPLAPSSKSTSGGTAALGCLVKDYFPEPVTVSWNSGALTSGVHTFPAVLQSSGLYSLSSVVTVPSSSLGTQTYICNVNHKPSNTKVDKKVEPKSCDKTHTCPPCPAPELLGGPSVFLFPPKPKDTLMISRTPEVTCVVVDVSHEDPEVKFNWYVDGVEVHNAKTKPREEQYNSTYRVVSVLTVLHQDWLNGKEYKCKVSNKALPAPIEKTISKAKGQPREPQVYTLPPSRDELTKNQVSLTCLVKGFYPSDIAVEWESNGQPENNYKTTPPVLDSDGSFFLYSKLTVDKSRWQQGNVFSCSVMHEALHNHYTQKSLSLSPGK

SEQ ID NO: 90 - DNA, 321 bp, Homo sapian
gacatccagatgacccagtctccatcttccgtgtctgcatctgtaggagacagagtcaccatcacttgtcgggcgagtcagggtattagcaggtggttagcctggtatcagcagaaaccagggaaagcccctaagctcctgatctatgctgcatccagtttgcaaagtggggtcccatcaaggttcagcggcagtggatctgggacagatttcactctcaccatcagcagcctgcagcctgaagattttgcaacttattactgtcagcaggcattctcccacccttggacttttggcggagggaccaaggttgagatcaaa

SEQ ID NO: 91 - protein, 107 aa, Homo sapian
DIQMTQSPSSVSASVGDRVTITCRASQGISRWLAWYQQKPGKAPKLLIYAASSLQSGVPSRFSGSGSGTDFTLTISSLQPEDFATYYCQQAFSHPWTFGGGTKVEIK

SEQ ID NO: 92 - protein, 11 aa, Homo sapian
RASQGISRWLA

SEQ ID NO: 93 - protein, 6 aa, Homo sapian
ASSLQS

SEQ ID NO: 94 - protein, 9 aa, Homo sapian
QQAFSHPWT

SEQ ID NO: 95 - DNA, 642 bp, Homo sapian
gacatccagatgacccagtctccatcttccgtgtctgcatctgtaggagacagagtcaccatcacttgtcgggcgagtcagggtattagcaggtggttagcctggtatcagcagaaaccagggaaagcccctaagctcctgatctatgctgcatccagtttgcaaagtggggtcccatcaaggttcagcggcagtggatctgggacagatttcactctcaccatcagcagcctgcagcctgaagattttgcaacttattactgtcagcaggcattctcccacccttggacttttggcggagggaccaaggttgagatcaaacgtacggtggctgcaccttccgtctttatctttccaccttccgatgagcagctgaagagcggaacagcaagcgtggtgtgtctgctgaacaacttttatccccgggaggcaaaggtgcagtggaaagtcgacaatgctctccagtccggcaattcccaagagagcgtgacagagcaagattccaaggactccacttacagcctgtccagcaccctcacactgagcaaggctgattacgagaaacacaaagtgtacgcttgtgaagtcacccaccaaggcctgagcagcccagtcactaagtcctttaaccggggcgaatgt

SEQ ID NO: 96 - protein, 107 aa, Homo sapian; identical to SEQ ID NO: 91

SEQ ID NO: 97 - DNA, 360 bp, Homo sapian
caggtgcagctggtgcagtctggggctgaggtgaagaagcctggggcctcagtgaaggtctcctgcaaggcttctggatacaccttcaccggccataagatgcactgggtgcgacaggcccctggacaagggcttgagtggatgggatggatcaaccctgctagtggttggacaaactatgcacagaagtttcagggcagggtcaccatgaccagggacacgtccatcagcacagcctacatggagctgagcaggctgagatctgacgacacggcggtgtactactgcgccagagtatctatgtacgccccagagccaatggacgtatggggccagggaacaactgtcaccgtctcctca

SEQ ID NO: 98 - protein, 120 aa, Homo sapian
QVQLVQSGAEVKKPGASVKVSCKASGYTFTGHKMHWVRQAPGQGLEWMGWINPASGWTNYAQKFQGRVTMTRDTSISTAYMELSRLRSDDTAVYYCARVSMYAPEPMDVWGQGTTVTVSS

SEQ ID NO: 99 - protein, 10 aa, Homo sapian
GYTFTGHKMH

SEQ ID NO: 100 - protein, 6 aa, Homo sapian
NPASGW

SEQ ID NO: 101 - protein, 11 aa, Homo sapian
VSMYAPEPMDV

SEQ ID NO: 102 - DNA, 1350 bp, Homo sapian
caggtgcagctggtgcagtctggggctgaggtgaagaagcctggggcctcagtgaaggtctcctgcaaggcttctggatacaccttcaccggccataagatgcactgggtgcgacaggcccctggacaagggcttgagtggatgggatggatcaaccctgctagtggttggacaaactatgcacagaagtttcagggcagggtcaccatgaccagggacacgtccatcagcacagcctacatggagctgagcaggctgagatctgacgacacggcggtgtactactgcgccagagtatctatgtacgccccagagccaatggacgtatggggccagggaacaactgtcaccgtctcctcagctagcacaaaaggaccaagcgtgtttccactggcacctagcagcaaatccaccagcggcggaacagcagccctcgggtgcctggtgaaggattacttccctgagccagtcacagtgtcctggaactccggagccctgacatccggcgtgcacaccttccccgctgtgctgcaatccagcggactgtatagcctcagctccgtcgtgacagtcccttccagcagcctgggcacacagacttacatttgcaacgtgaaccacaaaccttccaacactaaggtggacaaaaaggtggaacccaaatcctgtgataagacccatacatgcccaccttgtcccgctcctgagctgctggggggaccttccgtctttctgtttcctccaaaaccaaaagacacactcatgatcagccggacccccgaagtcacctgtgtggtggtggacgtcagccacgaagatccagaggtcaagttcaattggtacgtggatggagtggaagtccacaacgcaaaaaccaaacctagagaagaacagtacaatagcacatacagggtggtgtccgtcctgacagtgctccaccaggactggctcaatggcaaagagtataagtgcaaggtgagcaacaaggccctgcctgcaccaattgagaaaacaattagcaaggcaaaggggcagccacgggaaccccaggtgtataccctgcccccaagccgggatgaactgaccaaaaaccaggtcagcctgacatgcctggtgaaagggttttacccaagcgatattgccgtcgagtgggagagcaacggacagccagaaaacaattacaaaaccaccccacctgtgctggactccgatgggagctttttcctgtacagcaagctcacagtggacaagtccagatggcaacagggcaacgtgttttcctgctccgtgatgcacgaggccctccacaaccactatacacaaaagtccctctccctcagcccaggaaag

SEQ ID NO: 103 - protein, 450 aa, Homo sapian
QVQLVQSGAEVKKPGASVKVSCKASGYTFTGHKMHWVRQAPGQGLEWMGWINPASGWTNYAQKFQGRVTMTRDTSISTAYMELSRLRSDDTAVYYCARVSMYAPEPMDVWGQGTTVTVSSASTKGPSVFPLAPSSKSTSGGTAALGCLVKDYFPEPVTVSWNSGALTSGVHTFPAVLQSSGLYSLSSVVTVPSSSLGTQTYICNVNHKPSNTKVDKKVEPKSCDKTHTCPPCPAPELLGGPSVFLFPPKPKDTLMISRTPEVTCVVVDVSHEDPEVKFNWYVDGVEVHNAKTKPREEQYNSTYRVVSVLTVLHQDWLNGKEYKCKVSNKALPAPIEKTISKAKGQPREPQVYTLPPSRDELTKNQVSLTCLVKGFYPSDIAVEWESNGQPENNYKTTPPVLDSDGSFFLYSKLTVDKSRWQQGNVFSCSVMHEALHNHYTQKSLSLSPGK

SEQ ID NO: 104 - DNA, 360 bp, Homo sapian
caggtgcagctggtgcagtctggggctgaggtgaagaagcctggggcctcagtgaaggtttcctgcaaggcatctggatacaccttcaccagctacaatatggcgtgggtgcgacaggcccctggacaagggcttgagtggatgggaataatcaggcctagtgttggtagcacaagctacgcacagaagttccagggcagagtcaccatgaccagggacacgtccacgagcacagtctacatggagctgagcagcctgagatctgaggacacggcggtgtactactgcgctagagtatctatgtacgccccagagccaatggacgtatggggccagggaacaactgtcaccgtctcctca

SEQ ID NO: 105 - protein, 120 aa, Homo sapian
QVQLVQSGAEVKKPGASVKVSCKASGYTFTSYNMAWVRQAPGQGLEWMGIIRPSVGSTSYAQKFQGRVTMTRDTSTSTVYMELSSLRSEDTAVYYCARVSMYAPEPMDVWGQGTTVTVSS

SEQ ID NO: 106 - protein, 7 aa, Homo sapian
GYTFTSY

SEQ ID NO: 107 - protein, 6 aa, Homo sapian
RPSVGS

SEQ ID NO: 108 - protein, 11 aa, Homo sapian
VSMYAPEPMDV

SEQ ID NO: 109 - DNA, 1350 bp, Homo sapian
caggtgcagctggtgcagtctggggctgaggtgaagaagcctggggcctcagtgaaggtttcctgcaaggcatctggatacaccttcaccagctacaatatggcgtgggtgcgacaggcccctggacaagggcttgagtggatgggaataatcaggcctagtgttggtagcacaagctacgcacagaagttccagggcagagtcaccatgaccagggacacgtccacgagcacagtctacatggagctgagcagcctgagatctgaggacacggcggtgtactactgcgctagagtatctatgtacgccccagagccaatggacgtatggggccagggaacaactgtcaccgtctcctcagctagcacaaaaggaccaagcgtgtttccactggcacctagcagcaaatccaccagcggcggaacagcagccctcgggtgcctggtgaaggattacttccctgagccagtcacagtgtcctggaactccggagccctgacatccggcgtgcacaccttccccgctgtgctgcaatccagcggactgtatagcctcagctccgtcgtgacagtcccttccagcagcctgggcacacagacttacatttgcaacgtgaaccacaaaccttccaacactaaggtggacaaaaaggtggaacccaaatcctgtgataagacccatacatgcccaccttgtcccgctcctgagctgctggggggaccttccgtctttctgtttcctccaaaaccaaaagacacactcatgatcagccggacccccgaagtcacctgtgtggtggtggacgtcagccacgaagatccagaggtcaagttcaattggtacgtggatggagtggaagtccacaacgcaaaaaccaaacctagagaagaacagtacaatagcacatacagggtggtgtccgtcctgacagtgctccaccaggactggctcaatggcaaagagtataagtgcaaggtgagcaacaaggccctgcctgcaccaattgagaaaacaattagcaaggcaaaggggcagccacgggaaccccaggtgtataccctgcccccaagccgggatgaactgaccaaaaaccaggtcagcctgacatgcctggtgaaagggttttacccaagcgatattgccgtcgagtgggagagcaacggacagccagaaaacaattacaaaaccaccccacctgtgctggactccgatgggagctttttcctgtacagcaagctcacagtggacaagtccagatggcaacagggcaacgtgttttcctgctccgtgatgcacgaggccctccacaaccactatacacaaaagtccctctccctcagcccaggaaag

SEQ ID NO: 110 - protein, 450 aa, Homo sapian
QVQLVQSGAEVKKPGASVKVSCKASGYTFTSYNMAWVRQAPGQGLEWMGIIRPSVGSTSYAQKFQGRVTMTRDTSTSTVYMELSSLRSEDTAVYYCARVSMYAPEPMDVWGQGTTVTVSSASTKGPSVFPLAPSSKSTSGGTAALGCLVKDYFPEPVTVSWNSGALTSGVHTFPAVLQSSGLYSLSSVVTVPSSSLGTQTYICNVNHKPSNTKVDKKVEPKSCDKTHTCPPCPAPELLGGPSVFLFPPKPKDTLMISRTPEVTCVVVDVSHEDPEVKFNWYVDGVEVHNAKTKPREEQYNSTYRVVSVLTVLHQDWLNGKEYKCKVSNKALPAPIEKTISKAKGQPREPQVYTLPPSRDELTKNQVSLTCLVKGFYPSDIAVEWESNGQPENNYKTTPPVLDSDGSFFLYSKLTVDKSRWQQGNVFSCSVMHEALHNHYTQKSLSLSPGK

SEQ ID NO: 111 - DNA, 360 bp, Homo sapian
caggtgcagctggtgcagtctggggctgaggtgaagaagcctggggcctcagtgaaggtttcctgcaaggcatctggatacaccttcacctcgtaccgtatgcactgggtgcgacaggcccctggacaagggcttgagtggatgggatttatcgtgcctagtggtggtagcacaagctacgcacagaagttccagggcagagtcaccatgaccagggacacgtccacgagcacagtctacatggagctgagcagcctgagatctgaggacacggcggtgtactactgcgctagagtatctatgtacgccccagagccaatggacgtatggggccagggaacaactgtcaccgtctcctca

SEQ ID NO: 112 - protein, 120 aa, Homo sapian
QVQLVQSGAEVKKPGASVKVSCKASGYTFTSYRMHWVRQAPGQGLEWMGFIVPSGGSTSYAQKFQGRVTMTRDTSTSTVYMELSSLRSEDTAVYYCARVSMYAPEPMDVWGQGTTVTVSS

SEQ ID NO: 113 - protein, 7 aa, Homo sapian
GYTFTSY

SEQ ID NO: 114 - protein, 6 aa, Homo sapian
VPSGGS

SEQ ID NO: 115 - protein, 11 aa, Homo sapian
VSMYAPEPMDV

SEQ ID NO: 116 - DNA, 1350 bp, Homo sapian
caggtgcagctggtgcagtctggggctgaggtgaagaagcctggggcctcagtgaaggtttcctgcaaggcatctggatacaccttcacctcgtaccgtatgcactgggtgcgacaggcccctggacaagggcttgagtggatgggatttatcgtgcctagtggtggtagcacaagctacgcacagaagttccagggcagagtcaccatgaccagggacacgtccacgagcacagtctacatggagctgagcagcctgagatctgaggacacggcggtgtactactgcgctagagtatctatgtacgccccagagccaatggacgtatggggccagggaacaactgtcaccgtctcctcagctagcacaaaaggaccaagcgtgtttccactggcacctagcagcaaatccaccagcggcggaacagcagccctcgggtgcctggtgaaggattacttccctgagccagtcacagtgtcctggaactccggagccctgacatccggcgtgcacaccttccccgctgtgctgcaatccagcggactgtatagcctcagctccgtcgtgacagtcccttccagcagcctgggcacacagacttacatttgcaacgtgaaccacaaaccttccaacactaaggtggacaaaaaggtggaacccaaatcctgtgataagacccatacatgcccaccttgtcccgctcctgagctgctggggggaccttccgtctttctgtttcctccaaaaccaaaagacacactcatgatcagccggacccccgaagtcacctgtgtggtggtggacgtcagccacgaagatccagaggtcaagttcaattggtacgtggatggagtggaagtccacaacgcaaaaaccaaacctagagaagaacagtacaatagcacatacagggtggtgtccgtcctgacagtgctccaccaggactggctcaatggcaaagagtataagtgcaaggtgagcaacaaggccctgcctgcaccaattgagaaaacaattagcaaggcaaaggggcagccacgggaaccccaggtgtataccctgcccccaagccgggatgaactgaccaaaaaccaggtcagcctgacatgcctggtgaaagggttttacccaagcgatattgccgtcgagtgggagagcaacggacagccagaaaacaattacaaaaccaccccacctgtgctggactccgatgggagctttttcctgtacagcaagctcacagtggacaagtccagatggcaacagggcaacgtgttttcctgctccgtgatgcacgaggccctccacaaccactatacacaaaagtccctctccctcagcccaggaaag

SEQ ID NO: 117 - protein, 450 aa, Homo sapian
QVQLVQSGAEVKKPGASVKVSCKASGYTFTSYRMHWVRQAPGQGLEWMGFIVPSGGSTSYAQKFQGRVTMTRDTSTSTVYMELSSLRSEDTAVYYCARVSMYAPEPMDVWGQGTTVTVSSASTKGPSVFPLAPSSKSTSGGTAALGCLVKDYFPEPVTVSWNSGALTSGVHTFPAVLQSSGLYSLSSVVTVPSSSLGTQTYICNVNHKPSNTKVDKKVEPKSCDKTHTCPPCPAPELLGGPSVFLFPPKPKDTLMISRTPEVTCVVVDVSHEDPEVKFNWYVDGVEVHNAKTKPREEQYNSTYRVVSVLTVLHQDWLNGKEYKCKVSNKALPAPIEKTISKAKGQPREPQVYTLPPSRDELTKNQVSLTCLVKGFYPSDIAVEWESNGQPENNYKTTPPVLDSDGSFFLYSKLTVDKSRWQQGNVFSCSVMHEALHNHYTQKSLSLSPGK

SEQ ID NO: 118 - DNA, 360 bp, Homo sapian
caggtgcagctggtgcagtctggggctgaggtgaagaagcctggggcctcagtgaaggtttcctgcaaggcatctggatacaccttcacctcgtaccgtatgcactgggtgcgacaggcccctggacaagggcttgagtggatgggatttatcgtgcctagtggtggtagcacaggctacgcacagaagttccagggcagagttaccatgaccagggacacgtccacgagcacagtctacatggagctgagcagcctgagatctgaggacacggcggtgtactactgcgctagagtatctaggtacgccccagagccaatggacgtatggggccagggaacaactgtcaccgtctcctca

SEQ ID NO: 119 - protein, 120 aa, Homo sapian
QVQLVQSGAEVKKPGASVKVSCKASGYTFTSYRMHWVRQAPGQGLEWMGFIVPSGGSTGYAQKFQGRVTMTRDTSTSTVYMELSSLRSEDTAVYYCARVSRYAPEPMDVWGQGTTVTVSS

SEQ ID NO: 120 - protein, 6 aa, Homo sapian
VPSGGS

SEQ ID NO: 121 - protein, 11 aa, Homo sapian
VSRYAPEPMDV

SEQ ID NO: 122 - DNA, 1350 bp, Homo sapian
caggtgcagctggtgcagtctggggctgaggtgaagaagcctggggcctcagtgaaggtttcctgcaaggcatctggatacaccttcacctcgtaccgtatgcactgggtgcgacaggcccctggacaagggcttgagtggatgggatttatcgtgcctagtggtggtagcacaggctacgcacagaagttccagggcagagttaccatgaccagggacacgtccacgagcacagtctacatggagctgagcagcctgagatctgaggacacggcggtgtactactgcgctagagtatctaggtacgccccagagccaatggacgtatggggccagggaacaactgtcaccgtctcctcagctagcacaaaaggaccaagcgtgtttccactggcacctagcagcaaatccaccagcggcggaacagcagccctcgggtgcctggtgaaggattacttccctgagccagtcacagtgtcctggaactccggagccctgacatccggcgtgcacaccttccccgctgtgctgcaatccagcggactgtatagcctcagctccgtcgtgacagtcccttccagcagcctgggcacacagacttacatttgcaacgtgaaccacaaaccttccaacactaaggtggacaaaaaggtggaacccaaatcctgtgataagacccatacatgcccaccttgtcccgctcctgagctgctggggggaccttccgtctttctgtttcctccaaaaccaaaagacacactcatgatcagccggacccccgaagtcacctgtgtggtggtggacgtcagccacgaagatccagaggtcaagttcaattggtacgtggatggagtggaagtccacaacgcaaaaaccaaacctagagaagaacagtacaatagcacatacagggtggtgtccgtcctgacagtgctccaccaggactggctcaatggcaaagagtataagtgcaaggtgagcaacaaggccctgcctgcaccaattgagaaaacaattagcaaggcaaaggggcagccacgggaaccccaggtgtataccctgcccccaagccgggatgaactgaccaaaaaccaggtcagcctgacatgcctggtgaaagggttttacccaagcgatattgccgtcgagtgggagagcaacggacagccagaaaacaattacaaaaccaccccacctgtgctggactccgatgggagctttttcctgtacagcaagctcacagtggacaagtccagatggcaacagggcaacgtgttttcctgctccgtgatgcacgaggccctccacaaccactatacacaaaagtccctctccctcagcccaggaaag

SEQ ID NO: 123 - protein, 450 aa, Homo sapiens
QVQLVQSGAEVKKPGASVKVSCKASGYTFTSYRMHWVRQAPGQGLEWMGFIVPSGGSTGYAQKFQGRVTMTRDTSTSTVYMELSSLRSEDTAVYYCARVSRYAPEPMDVWGQGTTVTVSSASTKGPSVFPLAPSSKSTSGGTAALGCLVKDYFPEPVTVSWNSGALTSGVHTFPAVLQSSGLYSLSSVVTVPSSSLGTQTYICNVNHKPSNTKVDKKVEPKSCDKTHTCPPCPAPELLGGPSVFLFPPKPKDTLMISRTPEVTCVVVDVSHEDPEVKFNWYVDGVEVHNAKTKPREEQYNSTYRVVSVLTVLHQDWLNGKEYKCKVSNKALPAPIEKTISKAKGQPREPQVYTLPPSRDELTKNQVSLTCLVKGFYPSDIAVEWESNGQPENNYKTTPPVLDSDGSFFLYSKLTVDKSRWQQGNVFSCSVMHEALHNHYTQKSLSLSPGK

SEQ ID NO: 124 - DNA, 366 bp, Homo sapian
caggtgcagctgcaggagtcgggcccaggactggtgaagccttcacagaccctgtccctcacctgtactgtctctggtggctccatcagcagtggtagctactactggagctggatccgccagcacccagggaagggcctggagtggattgggtacatctattacagtgggagcacctactacaacccgtccctcaagagtcgagttaccatatcagtagacacgtctaagaaccagttctccctgaagctgagttctgtgaccgccgcagacacggcggtgtactactgcgccagaggactaggaatgtactaccacgtgccattcgacatatggggtcagggtacaatggtcaccgtctcctca

SEQ ID NO: 125 - protein, 122 aa, Homo sapian
QVQLQESGPGLVKPSQTLSLTCTVSGGSISSGSYYWSWIRQHPGKGLEWIGYIYYSGSTYYNPSLKSRVTISVDTSKNQFSLKLSSVTAADTAVYYCARGLGMYYHVPFDIWGQGTMVTVSS

SEQ ID NO: 126 - protein, 9 aa, Homo sapian
GGSISSGSY

SEQ ID NO: 127 - protein, 5 aa, Homo sapian
YYSGS

SEQ ID NO: 128 - protein, 12 aa, Homo sapian
GLGMYYHVPFDI

SEQ ID NO: 129 - DNA, 1356 bp, Homo sapian
caggtgcagctgcaggagtcgggcccaggactggtgaagccttcacagaccctgtccctcacctgtactgtctctggtggctccatcagcagtggtagctactactggagctggatccgccagcacccagggaagggcctggagtggattgggtacatctattacagtgggagcacctactacaacccgtccctcaagagtcgagttaccatatcagtagacacgtctaagaaccagttctccctgaagctgagttctgtgaccgccgcagacacggcggtgtactactgcgccagaggactaggaatgtactaccacgtgccattcgacatatggggtcagggtacaatggtcaccgtctcctcagctagcacaaaaggaccaagcgtgtttccactggcacctagcagcaaatccaccagcggcggaacagcagccctcgggtgcctggtgaaggattacttccctgagccagtcacagtgtcctggaactccggagccctgacatccggcgtgcacaccttccccgctgtgctgcaatccagcggactgtatagcctcagctccgtcgtgacagtcccttccagcagcctgggcacacagacttacatttgcaacgtgaaccacaaaccttccaacactaaggtggacaaaaaggtggaacccaaatcctgtgataagacccatacatgcccaccttgtcccgctcctgagctgctggggggaccttccgtctttctgtttcctccaaaaccaaaagacacactcatgatcagccggacccccgaagtcacctgtgtggtggtggacgtcagccacgaagatccagaggtcaagttcaattggtacgtggatggagtggaagtccacaacgcaaaaaccaaacctagagaagaacagtacaatagcacatacagggtggtgtccgtcctgacagtgctccaccaggactggctcaatggcaaagagtataagtgcaaggtgagcaacaaggccctgcctgcaccaattgagaaaacaattagcaaggcaaaggggcagccacgggaaccccaggtgtataccctgcccccaagccgggatgaactgaccaaaaaccaggtcagcctgacatgcctggtgaaagggttttacccaagcgatattgccgtcgagtgggagagcaacggacagccagaaaacaattacaaaaccaccccacctgtgctggactccgatgggagctttttcctgtacagcaagctcacagtggacaagtccagatggcaacagggcaacgtgttttcctgctccgtgatgcacgaggccctccacaaccactatacacaaaagtccctctccctcagcccaggaaag

SEQ ID NO: 130 - protein, 452 aa, Homo sapian
QVQLQESGPGLVKPSQTLSLTCTVSGGSISSGSYYWSWIRQHPGKGLEWIGYIYYSGSTYYNPSLKSRVTISVDTSKNQFSLKLSSVTAADTAVYYCARGLGMYYHVPFDIWGQGTMVTVSSASTKGPSVFPLAPSSKSTSGGTAALGCLVKDYFPEPVTVSWNSGALTSGVHTFPAVLQSSGLYSLSSVVTVPSSSLGTQTYICNVNHKPSNTKVDKKVEPKSCDKTHTCPPCPAPELLGGPSVFLFPPKPKDTLMISRTPEVTCVVVDVSHEDPEVKFNWYVDGVEVHNAKTKPREEQYNSTYRVVSVLTVLHQDWLNGKEYKCKVSNKALPAPIEKTISKAKGQPREPQVYTLPPSRDELTKNQVSLTCLVKGFYPSDIAVEWESNGQPENNYKTTPPVLDSDGSFFLYSKLTVDKSRWQQGNVFSCSVMHEALHNHYTQKSLSLSPGK

SEQ ID NO: 131 - DNA, 321 bp, Homo sapian
gaaattgtgttgacacagtctccagccaccctgtctttgtctccaggggaaagagccaccctctcctgcagggccagtcagagtgttagcagctacttagcctggtaccaacagaaacctggccaggctcccaggctcctcatctatgatgcatccaacagggccactggcatcccagccaggttcagtggcagtgggtctgggacagacttcactctcaccatcagcagcctagagcctgaagattttgcagtttattactgtcagcagtacttccactggcctcctacttttggcggagggaccaaggttgagatcaaa

SEQ ID NO: 132 - protein, 107 aa, Homo sapian
EIVLTQSPATLSLSPGERATLSCRASQSVSSYLAWYQQKPGQAPRLLIYDASNRATGIPARFSGSGSGTDFTLTISSLEPEDFAVYYCQQYFHWPPTFGGGTKVEIK

SEQ ID NO: 133 - protein, 11 aa, Homo sapian
RASQSVSSYLA

SEQ ID NO: 134 - protein, 7 aa, Homo sapian
DASNRAT

SEQ ID NO: 135 - protein, 9 aa, Homo sapian
QQYFHWPPT

SEQ ID NO: 136 - DNA, 642 bp, Homo sapian
gaaattgtgttgacacagtctccagccaccctgtctttgtctccaggggaaagagccaccctctcctgcagggccagtcagagtgttagcagctacttagcctggtaccaacagaaacctggccaggctcccaggctcctcatctatgatgcatccaacagggccactggcatcccagccaggttcagtggcagtgggtctgggacagacttcactctcaccatcagcagcctagagcctgaagattttgcagtttattactgtcagcagtacttccactggcctcctacttttggcggagggaccaaggttgagatcaaacgtacggtggctgcaccttccgtctttatctttccaccttccgatgagcagctgaagagcggaacagcaagcgtggtgtgtctgctgaacaacttttatccccgggaggcaaaggtgcagtggaaagtcgacaatgctctccagtccggcaattcccaagagagcgtgacagagcaagattccaaggactccacttacagcctgtccagcaccctcacactgagcaaggctgattacgagaaacacaaagtgtacgcttgtgaagtcacccaccaaggcctgagcagcccagtcactaagtcctttaaccggggcgaatgt

SEQ ID NO: 137 - protein, 214 aa, Homo sapian
EIVLTQSPATLSLSPGERATLSCRASQSVSSYLAWYQQKPGQAPRLLIYDASNRATGIPARFSGSGSGTDFTLTISSLEPEDFAVYYCQQYFHWPPTFGGGTKVEIKRTVAAPSVFIFPPSDEQLKSGTASVVCLLNNFYPREAKVQWKVDNALQSGNSQESVTEQDSKDSTYSLSSTLTLSKADYEKHKVYACEVTHQGLSSPVTKSFNRGEC

SEQ ID NO: 138 - protein, 118 aa, Homo sapian
ILGRSETQECLFFNANWEKDRTNQTGVEPCYGDKDKRRHCFATWKNISGSIEIVKQGCWLDDINCYDRTDCVEKKDSPEVYFCCCEGNMCNEKFSYFPEMEVTQPTSNPVTPKPPYYN

SEQ ID NO: 139 - protein, 106 aa, Homo sapian
ETRECIYYNANWELERTNQSGLERCEGEQDKRLHCYASWRNSSGTIELVKKGCWLDDFNCYDRQECVATEENPQVYFCCCEGNFCNERFTHLPEAGGPEVTYEPPP

SEQ ID NO: 140 - protein, 9 aa, Artificial Sequence
  human antigen binding domain of DO3 antibody
YTFTSYRMH

SEQ ID NO: 141 - protein, 17 aa, Artificial Sequence
  human antigen binding domain of DO3 antibody
FIVPSGGSTGYAQKFQG

SEQ ID NO: 142 - protein, 13 aa, Artificial Sequence
  human antigen binding domain of DO3 antibody
ARVSRYAPEPMDV

SEQ ID NO: 143 - DNA, 354 bp, Artificial Sequence
  VH sequence
gaggtgcagctgttggagtctgggggaggcttggtacagcctggggggtccctgagactctcctgtgcagcctctggattcacctttgggagctatggcatgacttgggtccgccaggctccagggaaggggctggagtgggtctcagttattagtggaagtggtggtgggacatactacgcagactccgtgaagggccggttcaccatctccagagacaattccaagaacacgctgtatctgcaaatgaacagcctgagagccgaggacacggcggtgtactactgcgccaagggtcctagaatagtgggcatggatgtgtggggccagggaacaactgtcaccgtctcctca

SEQ ID NO: 144 - protein, 117 aa, Artificial Sequence
  VH sequence
EVQLLESGGGLVQPGGSLRLSCAASGFTFGSYGMTWVRQAPGKGLEWVSVISGSGGGTYYADSVKGRFTISRDNSKNTLYLQMNSLRAEDTAVYYCAKGPRIVGMDVWGQGTTVTVS

SEQ ID NO: 145 - protein, 5 aa, Artificial Sequence
  CDR1 amino acid residues 31-35 of SEQ ID NO 144
SYGMT

SEQ ID NO: 146 - protein, 17 aa, Artificial Sequence
  CDR2 amino acid residues 50-65 of SEQ ID NO 144
VISGSGGGTYYADSVKG

SEQ ID NO: 147 - protein, 9 aa, Artificial Sequence
  CDR3 amino acid residues 95-102 of SEQ ID NO 144
GPRIVGMDV

SEQ ID NO: 148 - DNA, 1338 bp, Artificial Sequence
  H sequence
gaggtgcagctgttggagtctgggggaggcttggtacagcctggggggtccctgagactctcctgtgcagcctctggattcacctttgggagctatggcatgacttgggtccgccaggctccagggaaggggctggagtgggtctcagttattagtggaagtggtggtgggacatactacgcagactccgtgaagggccggttcaccatctccagagacaattccaagaacacgctgtatctgcaaatgaacagcctgagagccgaggacacggcggtgtactactgcgccaagggtcctagaatagtgggcatggatgtgtggggccagggaacaactgtcaccgtctcctcagcttccaccaagggcccatccgtcttccccctggcgccctgctccaggagcacctccgagagcacagccgccctgggctgcctggtcaaggactacttccccgaaccggtgacggtgtcgtggaactcaggcgccctgaccagcggcgtgcacaccttcccggctgtcctacagtcctcaggactctactccctcagcagcgtggtgaccgtgccctccagcagcttgggcacgaagacctacacctgcaacgtagatcacaagcccagcaacaccaaggtggacaagagagttgagtccaaatatggtcccccatgcccaccctgcccagcacctgagttcctggggggaccatcagtcttcctgttccccccaaaacccaaggacactctcatgatctcccggacccctgaggtcacgtgcgtggtggtggacgtgagccaggaagaccccgaggtccagttcaactggtacgtggatggcgtggaggtgcataatgccaagacaaagccgcgggaggagcagttcaacagcacgtaccgtgtggtcagcgtcctcaccgtcctgcaccaggactggctgaacggcaaggagtacaagtgcaaggtctccaacaaaggcctcccgtcctccatcgagaaaaccatctccaaagccaaagggcagccccgagagccacaggtgtacaccctgcccccatcccaggaggagatgaccaagaaccaggtcagcctgacctgcctggtcaaaggcttctaccccagcgacatcgccgtggagtgggagagcaatgggcagccggagaacaactacaagaccacgcctcccgtgctggactccgacggctccttcttcctctacagcaggctaaccgtggacaagagcaggtggcaggaggggaatgtcttctcatgctccgtgatgcatgaggctctgcacaaccactacacacagaagagcctctccctgtctctgggtaaatga

SEQ ID NO: 149 - protein, 445 aa, Artificial Sequence
  H sequence
EVQLLESGGGLVQPGGSLRLSCAASGFTFGSYGMTWVRQAPGKGLEWVSVISGSGGGTYYADSVKGRFTISRDNSKNTLYLQMNSLRAEDTAVYYCAKGPRIVGMDVWGQGTTVTVSSASTKGPSVFPLAPCSRSTSESTAALGCLVKDYFPEPVTVSWNSGALTSGVHTFPAVLQSSGLYSLSSVVTVPSSSLGTKTYTCNVDHKPSNTKVDKRVESKYGPPCPPCPAPEFLGGPSVFLFPPKPKDTLMISRTPEVTCVVVDVSQEDPEVQFNWYVDGVEVHNAKTKPREEQFNSTYRVVSVLTVLHQDWLNGKEYKCKVSNKGLPSSIEKTISKAKGQPREPQVYTLPPSQEEMTKNQVSLTCLVKGFYPSDIAVEWESNGQPENNYKTTPPVLDSDGSFFLYSRLTVDKSRWQEGNVFSCSVMHEALHNHYTQKSLSLSLGK

SEQ ID NO: 150 - DNA, 321 bp, Artificial Sequence
  VL sequence
gacatccagatgacccagtctccatcttccgtgtctgcatctgtaggagacagagtcaccatcacttgtcgggcgagtcagggtattagcagctggttagcctggtatcagcagaaaccagggaaagcccctaagctcctgatctatgctgcatccagtttgcaaagtggggtcccatcaaggttcagcggcagtggatctgggacagatttcactctcaccatcagcagcctgcagcctgaagattttgcaacttattactgtcagcaggtattcagttaccctctcacttttggcggagggaccaaggttgagatcaaa

SEQ ID NO: 151 - protein, 107 aa, Artificial Sequence
  VL sequence
DIQMTQSPSSVSASVGDRVTITCRASQGISSWLAWYQQKPGKAPKLLIYAASSLQSGVPSRFSGSGSGTDFTLTISSLQPEDFATYYCQQVFSYPLTFGGGTKVEIK

SEQ ID NO: 152 - protein, 11 aa, Artificial Sequence
  CDR1 amino acid residues 24-34 of SEQ ID NO 151
RASQGISSWLA

SEQ ID NO: 153 - protein, 7 aa, Artificial Sequence
  CDR2 amino acid residues 50-56 of SEQ ID NO 151
AASSLQS

SEQ ID NO: 154 - protein, 9 aa, Artificial Sequence
  CDR3 amino acid residues 89-97 of SEQ ID NO 151
QQVFSYPLT

SEQ ID NO: 155 - DNA, 645 bp, Artificial Sequence
  L sequence
gacatccagatgacccagtctccatcttccgtgtctgcatctgtaggagacagagtcaccatcacttgtcgggcgagtcagggtattagcagctggttagcctggtatcagcagaaaccagggaaagcccctaagctcctgatctatgctgcatccagtttgcaaagtggggtcccatcaaggttcagcggcagtggatctgggacagatttcactctcaccatcagcagcctgcagcctgaagattttgcaacttattactgtcagcaggtattcagttaccctctcacttttggcggagggaccaaggttgagatcaaacgaactgtggctgcaccatctgtcttcatcttcccgccatctgatgagcagttgaaatctggaactgcctctgttgtgtgcctgctgaataacttctatcccagagaggccaaagtacagtggaaggtggataacgccctccaatcgggtaactcccaggagagtgtcacagagcaggacagcaaggacagcacctacagcctcagcagcaccctgacgctgagcaaagcagactacgagaaacacaaagtctacgcctgcgaagtcacccatcagggcctgagctcgcccgtcacaaagagcttcaacaggggagagtgttag

SEQ ID NO: 156 - protein, 214 aa, Artificial Sequence
  L sequence
DIQMTQSPSSVSASVGDRVTITCRASQGISSWLAWYQQKPGKAPKLLIYAASSLQSGVPSRFSGSGSGTDFTLTISSLQPEDFATYYCQQVFSYPLTFGGGTKVEIKRTVAAPSVFIFPPSDEQLKSGTASVVCLLNNFYPREAKVQWKVDNALQSGNSQESVTEQDSKDSTYSLSSTLTLSKADYEKHKVYACEVTHQGLSSPVTKSFNRGEC

SEQ ID NO: 157 - protein, 9 aa, Artificial Sequence
  Peptide sequence of human ActRIIB
NANWELERT

SEQ ID NO: 158 - protein, 9 aa, Artificial Sequence
  Peptide sequence of human ActRIIB
VKKGCWLDD

SEQ ID NO: 159 - protein, 10 aa, Artificial Sequence
  Peptide sequence of human ActRIIB
CCEGNFCNER

SEQ ID NO: 160 - protein, 12 aa, Artificial Sequence
  Peptide sequence of human ActRIIB
GCWLDDFNCYDR

SEQ ID NO: 161 - protein, 10 aa, Artificial Sequence
  Peptide sequence of human ActRIIA
CCEGNMCNEK

SEQ ID NO: 162 - protein, 12 aa, Artificial Sequence
  Peptide sequence of human ActRIIA
ECLFFNANWEKD

SEQ ID NO: 163 - protein, 12 aa, Artificial Sequence
  Peptide sequence of human ActRIIA
CWLDDINCYDRT

SEQ ID NO: 164 - DNA, 360 bp, Artificial Sequence; identical to SEQ ID NO: 118
  VH sequence

SEQ ID NO: 165 - protein, 120 aa, Artificial Sequence; identical to SEQ ID NO: 119
  VH sequence

SEQ ID NO: 166 - protein, 5 aa, Artificial Sequence
  CDR1 amino acid residues 31-35 of SEQ ID NO 165
SYRMH

SEQ ID NO: 167 - protein, 17 aa, Artificial Sequence
  CDR2 amino acid residues 50-66 of SEQ ID NO 165
FIVPSGGSTGYAQKFQG

SEQ ID NO: 168 - protein, 11 aa, Artificial Sequence
  CDR3 amino acid residues 99-109 of SEQ ID NO 165
VSRYAPEPMDV

SEQ ID NO: 169 - DNA, 1344 bp, Artificial Sequence
  H sequence
caggtgcagctggtgcagtctggggctgaggtgaagaagcctggggcctcagtgaaggtttcctgcaaggcatctggatacaccttcacctcgtaccgtatgcactgggtgcgacaggcccctggacaagggcttgagtggatgggatttatcgtgcctagtggtggtagcacaggctacgcacagaagttccagggcagagttaccatgaccagggacacgtccacgagcacagtctacatggagctgagcagcctgagatctgaggacacggcggtgtactactgcgctagagtatctaggtacgccccagagccaatggacgtatggggccagggaacaactgtcaccgtctcctcagcttccaccaagggcccatccgtcttccccctggcgccctgctccaggagcacctccgagagcacagccgccctgggctgcctggtcaaggactacttccccgaaccggtgacggtgtcgtggaactcaggcgccctgaccagcggcgtgcacaccttcccggctgtcctacagtcctcaggactctactccctcagcagcgtggtgaccgtgccctccagcagcttgggcacgaagacctacacctgcaacgtagatcacaagcccagcaacaccaaggtggacaagagagttgagtccaaatatggtcccccatgcccaccctgcccagcacctgagttcctggggggaccatcagtcttcctgttccccccaaaacccaaggacactctcatgatctcccggacccctgaggtcacgtgcgtggtggtggacgtgagccaggaagaccccgaggtccagttcaactggtacgtggatggcgtggaggtgcataatgccaagacaaagccgcgggaggagcagttcaacagcacgtaccgtgtggtcagcgtcctcaccgtcctgcaccaggactggctgaacggcaaggagtacaagtgcaaggtctccaacaaaggcctcccgtcctccatcgagaaaaccatctccaaagccaaagggcagccccgagagccacaggtgtacaccctgcccccatcccaggaggagatgaccaagaaccaggtcagcctgacctgcctggtcaaaggcttctaccccagcgacatcgccgtggagtgggagagcaatgggcagccggagaacaactacaagaccacgcctcccgtgctggactccgacggctccttcttcctctacagcaggctaaccgtggacaagagcaggtggcaggaggggaatgtcttctcatgctccgtgatgcatgaggctctgcacaaccactacacacagaagagcctctccctgtctctgggtaaatga

SEQ ID NO: 170 - protein, 447 aa, Artificial Sequence
  H sequence
QVQLVQSGAEVKKPGASVKVSCKASGYTFTSYRMHWVRQAPGQGLEWMGFIVPSGGSTGYAQKFQGRVTMTRDTSTSTVYMELSSLRSEDTAVYYCARVSRYAPEPMDVWGQGTTVTVSSASTKGPSVFPLAPCSRSTSESTAALGCLVKDYFPEPVTVSWNSGALTSGVHTFPAVLQSSGLYSLSSVVTVPSSSLGTKTYTCNVDHKPSNTKVDKRVESKYGPPCPPCPAPEFLGGPSVFLFPPKPKDTLMISRTPEVTCVVVDVSQEDPEVQFNWYVDGVEVHNAKTKPREEQFNSTYRVVSVLTVLHQDWLNGKEYKCKVSNKGLPSSIEKTISKAKGQPREPQVYTLPPSQEEMTKNQVSLTCLVKGFYPSDIAVEWESNGQPENNYKTTPPVLDSDGSFFLYSRLTVDKSRWQEGNVFSCSVMHEALHNHYTQKSLSLSLGK

SEQ ID NO: 171 - DNA, 321 bp, Artificial Sequence; identical to SEQ ID NO: 90
  VL sequence

SEQ ID NO: 172 - protein, 107 aa, Artificial Sequence; identical to SEQ ID NO: 91
  VL sequence

SEQ ID NO: 173 - protein, 11 aa, Artificial Sequence
  CDR1 amino acid residues 24-34 of SEQ ID NO 172
RASQGISRWLA

SEQ ID NO: 174 - protein, 7 aa, Artificial Sequence
  CDR2 amino acid residues 50-56 of SEQ ID NO 172
AASSLQS

SEQ ID NO: 175 - protein, 9 aa, Artificial Sequence
  CDR3 amino acid residues 89-97 of SEQ ID NO 172
QQAFSHPWT

SEQ ID NO: 176 - DNA, 727 bp, Artificial Sequence
  L sequence
gacatccagatgacccagtctccatcttccgtgtctgcatctgtaggagacagagtcaccatcacttgtcgggcgagtcagggtattagcaggtggttagcctggtatcagcagaaaccagggaaagcccctaagctcctgatctatgctgcatccagtttgcaaagtggggtcccatcaaggttcagcggcagtggatctgggacagatttcactctcaccatcagcagcctgcagcctgaagattttgcaacttattactgtcagcaggcattctcccacccttggacttttggcggagggaccaaggttgagatcaaacgtaaggggctcacagttaattaattgaggtctggacatatacatgggtgacaatgacatccactttgcctttctctccacaggaactgtggctgcaccatctgtcttcatcttcccgccatctgatgagcagttgaaatctggaactgcctctgttgtgtgcctgctgaataacttctatcccagagaggccaaagtacagtggaaggtggataacgccctccaatcgggtaactcccaggagagtgtcacagagcaggacagcaaggacagcacctacagcctcagcagcaccctgacgctgagcaaagcagactacgagaaacacaaagtctacgcctgcgaagtcacccatcagggcctgagctcgcccgtcacaaagagcttcaacaggggagagtgttag

SEQ ID NO: 177 - protein, 214 aa, Artificial Sequence
  L sequence
DIQMTQSPSSVSASVGDRVTITCRASQGISRWLAWYQQKPGKAPKLLIYAASSLQSGVPSRFSGSGSGTDFTLTISSLQPEDFATYYCQQAFSHPWTFGGGTKVEIKRTVAAPSVFIFPPSDEQLKSGTASVVCLLNNFYPREAKVQWKVDNALQSGNSQESVTEQDSKDSTYSLSSTLTLSKADYEKHKVYACEVTHQGLSSPVTKSFNRGEC